European Patent Application EP 4 491 629 A1, published January 15, 2025. Title: EXPRESSION SYSTEM INCLUDING AN ENGINEERED LECTIN PROPERTY PURIFICATION TAG BASED ON CRICETULUS GRISEUS GALECTIN-1. Applicant: UNIVERSITE DE LORRAINE. The sequence listing filed with the application follows.

SEQUENCE LISTING (14 sequences)

SEQ ID NO: 1 - protein, 135 aa, synthetic construct
  VARIANT 19: note = X is K or R
  VARIANT 24: note = X is V or L
  VARIANT 26: note = X is P or S
  VARIANT 63: note = X is S or T
  VARIANT 65: note = X is D or E
  VARIANT 66: note = X is N, G, or D
  VARIANT 68: note = X is A or T
  VARIANT 73: note = X is H or Q
  VARIANT 76: note = X is P, A, or T
  VARIANT 77: note = X is A or V
  VARIANT 85: note = X is T, V, or I
  VARIANT 86: note = X is V, A or T
  VARIANT 96: note = X is D or N
  VARIANT 99: note = X is I or V
  VARIANT 105: note = X is H or Y
  VARIANT 115: note = X is M or L
  VARIANT 129: note = X is I or V
  VARIANT 131: note = X is a negatively charged amino acid, preferably is D or E, more preferably is E
  VARIANT 135: note = X is E or D
MACGLVASNLNLKPGECLXVRGEXAXDAKSFVLNLGKDSNNLCLHFNPRFNAHGDANTIVCNXKXXGXWGTEXREXXFPFQPGSXXEVCITFDQAXLTXKLPDGXEFKFPNRLNXEAINYMAADGDFKXKXVAFX

SEQ ID NO: 2 - protein, 135 aa, synthetic construct
MACGLVASNLNLKPGECLKVRGEVAPDAKSFVLNLGKDSNNLCLHFNPRFNAHGDANTIVCNSKDNGAWGTEHREPAFPFQPGSTVEVCITFDQADLTIKLPDGHEFKFPNRLNMEAINYMAADGDFKIKEVAFE

SEQ ID NO: 3 - protein, 135 aa, synthetic construct
MACGLVASNLNLKPGECLKVRGEVAPDAKSFVLNLGKDSNNLCLHFNPRFNAHGDANTIVCNSKDNGAWGTEHREPAFPFQPGSTVEVCITFDQADLTIKLPDGHEFKFPNRLNMEAINYMAADGDFKIKDVAFE

SEQ ID NO: 4 - DNA, 800 bp, synthetic construct
  source 1..800: mol_type = other DNA
  CDS 128..667: protein_id = 11; translation = MACGLVASNLNLKPGECLKVRGEVAPDAKSFVLNLGKDSNNLCLHFNPRFNAHGDANTIVCNSKDNGAWGTEHREPAFPFQPGSTVEVCITFDQADLTIKLPDGHEFKFPNRLNMEAINYMAADGDFKIKEVAFEELSSGVDLGTENLYFQSAMDINSDPNSSSVDKLAAALEHHHHHH
cccgtggccaggacccaacgctgcccgagatctcgatcccgcgaaattaatacgactcactatagggagaccacaacggtttccctctagaaataattttgtttaactttaagaaggagatatacatatggcatgtggtctggttgcaagcaatctgaatctgaaaccgggtgaatgtctgaaagttcgtggtgaagttgcaccggatgcaaaaagctttgtgctgaatctgggtaaagatagcaataatctgtgcctgcattttaaccctcgttttaatgcacatggtgatgccaataccattgtgtgcaatagcaaagataatggtgcatggggcaccgaacatcgtgaaccggcatttccgtttcagcctggtagcaccgttgaagtttgtattacctttgatcaggcagacctgaccattaaactgccggatggtcatgaattcaaatttccgaatcgtctgaatatggaagccatcaattatatggcagccgatggtgactttaagattaaagaagtggcctttgaagagctcagcagcggtgttgatctgggtacagaaaatctgtattttcagagcgccatggatatcaattcggatccgaattcgagctccgtcgacaagcttgcggccgcactcgagcaccaccaccaccaccactgagatccggctgctaacaaagcccgaaaggaagctgagttggctgctgccaccgctgagcaataactagcataaccccttggggcctctaaacgggtcttgaggggttttttgctgaaaggaggaactatatccg

SEQ ID NO: 5 - protein, 135 aa, synthetic construct
MACGLVASNLNLKPGKCLKVRGEVAPDAKSFVLNLGKDSNNLCLHFNPRFNAHGDANTIVCNSKDNGAWGTEHREPAFPFQPGSTVEVCITFDQADLTIKLPDGHEFKFPNRLNMEAINYMAADGDFKIKCVAFE

SEQ ID NO: 6 - protein, 135 aa, Cricetulus griseus
MACGLVASNLNLKPGECLKVRGEVAPDAKSFVLNLGKDSNNLCLHFNPRFNAHGDANTIVCNSKDNGAWGTEHREPAFPFQPGSTVEVCITFDQADLTIKLPDGHEFKFPNRLNMEAINYMAADGDFKIKCVAFE

SEQ ID NO: 7 - protein, 135 aa, Gorilla gorilla
MACGLVASNLNLKPGECLRVRGEVAPDAKSFVLNLGKDSNNLCLHFNPRFNAHGDANTIVCNSKDGGAWGTEQREAVFPFQPGSVAEVCITFDQANLTIKLPDGYEFKFPNRLNLEAINYMAADGDFKIKCVAFD

SEQ ID NO: 8 - protein, 135 aa, Homo sapiens
MACGLVASNLNLKPGECLRVRGEVAPDAKSFVLNLGKDSNNLCLHFNPRFNAHGDANTIVCNSKDGGAWGTEQREAVFPFQPGSVAEVCITFDQANLTVKLPDGYEFKFPNRLNLEAINYMAADGDFKIKCVAFD

SEQ ID NO: 9 - protein, 135 aa, Mus musculus
MACGLVASNLNLKPGECLKVRGEVASDAKSFVLNLGKDSNNLCLHFNPRFNAHGDANTIVCNTKEDGTWGTEHREPAFPFQPGSITEVXITFDQADLTIKLPDGHEFKFPNRLNMEAINYMAADGDFKIKCVAFE

SEQ ID NO: 10 - protein, 135 aa, Rattus rattus
MACGLVASNLNLKPGECLKVRGELAPDAKSFVLNLGKDSNNLCLHFNPRFNAHGDANTIVCNSKDDGTWGTEQRETAFPFQPGSITEVCITFDQADLTIKLPDGHEFKFPNRLNMEAINYMAADGDFKVKCVAFE

SEQ ID NO: 11 - protein, 179 aa, synthetic construct
MACGLVASNLNLKPGECLKVRGEVAPDAKSFVLNLGKDSNNLCLHFNPRFNAHGDANTIVCNSKDNGAWGTEHREPAFPFQPGSTVEVCITFDQADLTIKLPDGHEFKFPNRLNMEAINYMAADGDFKIKEVAFEELSSGVDLGTENLYFQSAMDINSDPNSSSVDKLAAALEHHHHHH

SEQ ID NO: 12 - protein, 13 aa, synthetic construct
ENLYFQSAMDINS

SEQ ID NO: 13 - protein, 10 aa, synthetic construct
ELSSGVDLGT

SEQ ID NO: 14 - protein, 7 aa, synthetic construct
ENLYFQS